European Patent Application EP 4 549 459 A1, published May 7, 2025. Title: AAV based agents for the treatment of neovascular-associated ocular fundus diseases. Applicant: SHANGHAI REFRESHGENE THERAPEUTICS CO.,LTD. The sequence listing filed with the application follows.

SEQUENCE LISTING (29 sequences)

SEQ ID NO: 1 - protein, 167 aa, synthetic construct
DGVEVHNAKTKPREEQYNSTYRVVSVLTVLAQDWLNGKEYKCKVSNKALPAPIEKTISKAKGQPREPQVYTLPPSRDELTKNQVSLTCLVKGFYPSDIAVEWESNGQPENNYKTTPPVLDSDGSFFLYSKLTVDKSRWQQGNVFSCSVMHEALHNHYTQKSLSLSPG

SEQ ID NO: 2 - protein, 167 aa, synthetic construct
DGVEVHNAKTKPREEQYNSTYRVVSVLTVLEQDWLNGKEYKCKVSNKALPAPIEKTISKAKGQPREPQVYTLPPSRDELTKNQVSLTCLVKGFYPSDIAVEWESNGQPENNYKTTPPVLDSDGSFFLYSKLTVDKSRWQQGNVFSCSVMHEALHNHYTQKSLSLSPG

SEQ ID NO: 3 - protein, 167 aa, synthetic construct
DGVEVHNAKTKPREEQYNSTYRVVSVLTVLHQDWLNGKEYKCKVSNKALPAPIEKTISKAKGQPREPQVYTLPPSRDELTKNQVSLTCLVKGFYPSDIAVEWESNGQPENNYKTTPPVLDSDGSFFLYSKLTVDKSRWQQGNVFSCSVMHEALHNAYTQKSLSLSPG

SEQ ID NO: 4 - protein, 167 aa, synthetic construct
DGVEVHNAKTKPREEQYNSTYRVVSVLTVLAQDWLNGKEYKCKVSNKALPAPIEKTISKAKGQPREPQVYTLPPSRDELTKNQVSLTCLVKGFYPSDIAVEWESNGQPENNYKTTPPVLDSDGSFFLYSKLTVDKSRWQQGNVFSCSVMHEALHNAYTQKSLSLSPG

SEQ ID NO: 5 - protein, 103 aa, Homo sapiens
SDTGRPFVEMYSEIPEIIHMTEGRELVIPCRVTSPNITVTLKKFPLDTLIPDGKRIIWDSRKGFIISNATYKEIGLLTCEATVNGHLYKTNYLTHRQTNTIID

SEQ ID NO: 6 - protein, 102 aa, Homo sapiens
VVLSPSHGIELSVGEKLVLNCTARTELNVGIDFNWEYPSSKHQHKKLVNRDLKTQSGSEMKKFLSTLTIDGVTRSDQGLYTCAASSGLMTKKNSTFVRVHEK

SEQ ID NO: 7 - protein, 431 aa, synthetic construct
SDTGRPFVEMYSEIPEIIHMTEGRELVIPCRVTSPNITVTLKKFPLDTLIPDGKRIIWDSRKGFIISNATYKEIGLLTCEATVNGHLYKTNYLTHRQTNTIIDVVLSPSHGIELSVGEKLVLNCTARTELNVGIDFNWEYPSSKHQHKKLVNRDLKTQSGSEMKKFLSTLTIDGVTRSDQGLYTCAASSGLMTKKNSTFVRVHEKDKTHTCPPCPAPELLGGPSVFLFPPKPKDTLMISRTPEVTCVVVDVSHEDPEVKFNWYVDGVEVHNAKTKPREEQYNSTYRVVSVLTVLAQDWLNGKEYKCKVSNKALPAPIEKTISKAKGQPREPQVYTLPPSRDELTKNQVSLTCLVKGFYPSDIAVEWESNGQPENNYKTTPPVLDSDGSFFLYSKLTVDKSRWQQGNVFSCSVMHEALHNHYTQKSLSLSPG

SEQ ID NO: 8 - protein, 431 aa, synthetic construct
SDTGRPFVEMYSEIPEIIHMTEGRELVIPCRVTSPNITVTLKKFPLDTLIPDGKRIIWDSRKGFIISNATYKEIGLLTCEATVNGHLYKTNYLTHRQTNTIIDVVLSPSHGIELSVGEKLVLNCTARTELNVGIDFNWEYPSSKHQHKKLVNRDLKTQSGSEMKKFLSTLTIDGVTRSDQGLYTCAASSGLMTKKNSTFVRVHEKDKTHTCPPCPAPELLGGPSVFLFPPKPKDTLMISRTPEVTCVVVDVSHEDPEVKFNWYVDGVEVHNAKTKPREEQYNSTYRVVSVLTVLEQDWLNGKEYKCKVSNKALPAPIEKTISKAKGQPREPQVYTLPPSRDELTKNQVSLTCLVKGFYPSDIAVEWESNGQPENNYKTTPPVLDSDGSFFLYSKLTVDKSRWQQGNVFSCSVMHEALHNHYTQKSLSLSPG

SEQ ID NO: 9 - protein, 431 aa, synthetic construct
SDTGRPFVEMYSEIPEIIHMTEGRELVIPCRVTSPNITVTLKKFPLDTLIPDGKRIIWDSRKGFIISNATYKEIGLLTCEATVNGHLYKTNYLTHRQTNTIIDVVLSPSHGIELSVGEKLVLNCTARTELNVGIDFNWEYPSSKHQHKKLVNRDLKTQSGSEMKKFLSTLTIDGVTRSDQGLYTCAASSGLMTKKNSTFVRVHEKDKTHTCPPCPAPELLGGPSVFLFPPKPKDTLMISRTPEVTCVVVDVSHEDPEVKFNWYVDGVEVHNAKTKPREEQYNSTYRVVSVLTVLHQDWLNGKEYKCKVSNKALPAPIEKTISKAKGQPREPQVYTLPPSRDELTKNQVSLTCLVKGFYPSDIAVEWESNGQPENNYKTTPPVLDSDGSFFLYSKLTVDKSRWQQGNVFSCSVMHEALHNAYTQKSLSLSPG

SEQ ID NO: 10 - protein, 431 aa, synthetic construct
SDTGRPFVEMYSEIPEIIHMTEGRELVIPCRVTSPNITVTLKKFPLDTLIPDGKRIIWDSRKGFIISNATYKEIGLLTCEATVNGHLYKTNYLTHRQTNTIIDVVLSPSHGIELSVGEKLVLNCTARTELNVGIDFNWEYPSSKHQHKKLVNRDLKTQSGSEMKKFLSTLTIDGVTRSDQGLYTCAASSGLMTKKNSTFVRVHEKDKTHTCPPCPAPELLGGPSVFLFPPKPKDTLMISRTPEVTCVVVDVSHEDPEVKFNWYVDGVEVHNAKTKPREEQYNSTYRVVSVLTVLAQDWLNGKEYKCKVSNKALPAPIEKTISKAKGQPREPQVYTLPPSRDELTKNQVSLTCLVKGFYPSDIAVEWESNGQPENNYKTTPPVLDSDGSFFLYSKLTVDKSRWQQGNVFSCSVMHEALHNAYTQKSLSLSPG

SEQ ID NO: 11 - protein, 686 aa, synthetic construct
DIQMTQSPSSLSASVGDRVTITCSASQDISNYLNWYQQKPGKAPKVLIYFTSSLHSGVPSRFSGSGSGTDFTLTISSLQPEDFATYYCQQYSTVPWTFGQGTKVEIKRTVAAPSVFIFPPSDEQLKSGTASVVCLLNNFYPREAKVQWKVDNALQSGNSQESVTEQDSKDSTYSLSSTLTLSKADYEKHKVYACEVTHQGLSSPVTKSFNRGECATNFSLLKQAGDVEENPGPEVQLVESGGGLVQPGGSLRLSCAASGYTFTNYGMNWVRQAPGKGLEWVGWINTYTGEPTYAADFKRRFTFSLDTSKSTAYLQMNSLRAEDTAVYYCAKYPHYYGSSHWYFDVWGQGTLVTVSSASTKGPSVFPLAPSSKSTSGGTAALGCLVKDYFPEPVTVSWNSGALTSGVHTFPAVLQSSGLYSLSSVVTVPSSSLGTQTYICNVNHKPSNTKVDKKVEPKSCDKTHTCPPCPAPELLGGPSVFLFPPKPKDTLMISRTPEVTCVVVDVSHEDPEVKFNWYVDGVEVHNAKTKPREEQYNSTYRVVSVLTVLEQDWLNGKEYKCKVSNKALPAPIEKTISKAKGQPREPQVYTLPPSREEMTKNQVSLTCLVKGFYPSDIAVEWESNGQPENNYKTTPPVLDSDGSFFLYSKLTVDKSRWQQGNVFSCSVMHEALHNHYTQKSLSLSPGK

SEQ ID NO: 12 - DNA, 5702 bp, synthetic construct
  source 1..5702: mol_type = other DNA
cctgcaggcagctgcgcgctcgctcgctcactgaggccgcccgggcaaagcccgggcgtcgggcgacctttggtcgcccggcctcagtgagcgagcgagcgcgcagagagggagtggccaactccatcactaggggttcctgcggccgcacgcgtggagctagttattaatagtaatcaattacggggtcattagttcatagcccatatatggagttccgcgttacataacttacggtaaatggcccgcctggctgaccgcccaacgacccccgcccattgacgtcaataatgacgtatgttcccatagtaacgtcaatagggactttccattgacgtcaatgggtggagtatttacggtaaactgcccacttggcagtacatcaagtgtatcatatgccaagtacgccccctattgacgtcaatgacggtaaatggcccgcctggcattatgcccagtacatgaccttatgggactttcctacttggcagtacatctacgtattagtcatcgctattaccatggtgatgcggttttggcagtacatcaatgggcgtggatagcggtttgactcacggggatttccaagtctccaccccattgacgtcaatgggagtttgttttgcaccaaaatcaacgggactttccaaaatgtcgtaacaactccgccccattgacgcaaatgggcggtaggcgtgtacggtgggaggtctatataagcagagctcgtttagtgaaccgtcagatcgcctggagacgccatccacgctgttttgacctccatagaagacaccgggaccgatccagcctccgcggattcgaatcccggccgggaacggtgcattggaacgcggattccccgtgccaagagtgacgtaagtaccgcctatagagtctataggcccacaaaaaatgctttcttcttttaatatacttttttgtttatcttatttctaatactttccctaatctctttctttcagggcaataatgatacaatgtatcatgcctctttgcaccattctaaagaataacagtgataatttctgggttaaggcaatagcaatatttctgcatataaatatttctgcatataaattgtaactgatgtaagaggtttcatattgctaatagcagctacaatccagctaccattctgcttttattttatggttgggataaggctggattattctgagtccaagctaggcccttttgctaatcatgttcatacctcttatcttcctcccacagctcctgggcaacgtgctggtctgtgtgctggcccatcactttggcaaagaattgggattcgaacatcgattgaattccccggggatcctctagagccgccaccatgggagtgaaagttctgttcgccctgatctgtatcgccgtggccgaggcctctgataccggcagacctttcgtggaaatgtacagcgagatccccgagatcatccacatgaccgagggcagagagctggtcatcccctgcagagtgacaagccccaacatcaccgtgactctgaagaagttccctctggacacactgatccccgacggcaagagaatcatctgggacagccggaagggcttcatcatcagcaacgccacctacaaagagatcggcctgctgacctgtgaagccaccgtgaatggccacctgtacaagaccaactacctgacacacagacagaccaacaccatcatcgacgtggtgctgagccctagccacggcattgaactgtctgtgggcgagaagctggtgctgaactgtaccgccagaaccgagctgaacgtgggcatcgacttcaactgggagtaccccagcagcaagcaccagcacaagaaactggtcaaccgggacctgaaaacccagagcggcagcgagatgaagaaattcctgagcaccctgaccatcgacggcgtgaccagatctgaccagggcctgtacacatgtgccgccagctctggcctgatgaccaagaaaaacagcaccttcgtgcgggtgcacgagaaggacaagacccacacctgtcctccatgtcctgctccagaactgctcggcggaccttccgtgttcctgtttcctccaaagcctaaggacaccctgatgatcagcagaacccctgaagtgacctgcgtggtggtggatgtgtctcacgaggaccccgaagtgaagttcaattggtacgtggacggcgtggaagtgcacaacgccaagaccaagcctagagaggaacagtacaatagcacctacagagtggtgtccgtgctgaccgtgctggagcaggattggctgaacggcaaagagtacaagtgcaaggtgtccaacaaggccctgcctgctcctatcgagaaaaccatctccaaggccaagggccagcctagggaaccccaggtttacacactgcctccaagcagggacgagctgacaaagaaccaggtgtccctgacctgcctggtcaagggcttctacccttccgacattgccgtggaatgggagagcaatggccagcctgagaacaactacaagacaacccctcctgtgctggacagcgacggctcattcttcctgtacagcaagctgacagtggacaagagcagatggcagcagggcaacgtgttcagctgctctgtgatgcacgaagccctgcacaaccactacacccagaagtccctgtctctgagccctggatgataaaagcttgcctcgagcagcgctgctcgagagatctacctgtgccttctagttgccagccatctgttgtttgcccctcccccgtgccttccttgaccctggaaggtgccactcccactgtcctttcctaataaaatgaggaaattgcatcgcattgtctgagtaggtgtcattctattctggggggtggggtggggcaggacagcaagggggaggattgggaagacaatagcaggcatgctggggatgcggtgggctctatggctgattttgtaggtaaccacgtgcggaccgagcggccgcaggaacccctagtgatggagttggccactccctctctgcgcgctcgctcgctcactgaggccgggcgaccaaaggtcgcccgacgcccgggctttgcccgggcggcctcagtgagcgagcgagcgcgcagctgcctgcaggggcgcctgatgcggtattttctccttacgcatctgtgcggtatttcacaccgcatacgtcaaagcaaccatagtacgcgccctgtagcggcgcattaagcgcggcgggtgtggtggttacgcgcagcgtgaccgctacacttgccagcgccctagcgcccgctcctttcgctttcttcccttcctttctcgccacgttcgccggctttccccgtcaagctctaaatcgggggctccctttagggttccgatttagtgctttacggcacctcgaccccaaaaaacttgatttgggtgatggttcacgtagtgggccatcgccctgatagacggtttttcgccctttgacgttggagtccacgttctttaatagtggactcttgttccaaactggaacaacactcaaccctatctcgggctattcttttgatttataagggattttgccgatttcggcctattggttaaaaaatgagctgatttaacaaaaatttaacgcgaattttaacaaaatattaacgtttacaattttatggtgcactctcagtacaatctgctctgatgccgcatagttaagccagccccgacacccgccaacacccgctgacgcgccctgacgggcttgtctgctcccggcatccgcttacagacaagctgtgaccgtctccgggagctgcatgtgtcagaggttttcaccgtcatcaccgaaacgcgcgagacgaaagggcctcgtgatacgcctatttttataggttaatgtcatgataataatggtttcttagacgtcaggtggcacttttcggggaaatgtgtgcagctctggcccgtgtctcaaaatctctgatgttacattgcacaagataaaaatatatcatcatgaacaataaaactgtctgcttacataaacagtaatacaaggggtgttatgagccatattcaacgggaaacgtcgaggccgcgattaaattccaacatggatgctgatttatatgggtataaatgggctcgcgataatgtcgggcaatcaggtgcgacaatctatcgcttgtatgggaagcccgatgcgccagagttgtttctgaaacatggcaaaggtagcgttgccaatgatgttacagatgagatggtcagactaaactggctgacggaatttatgcctcttccgaccatcaagcattttatccgtactcctgatgatgcatggttactcaccactgcgatccccggaaaaacagcattccaggtattagaagaatatcctgattcaggtgaaaatattgttgatgcgctggcagtgttcctgcgccggttgcattcgattcctgtttgtaattgtccttttaacagcgatcgcgtatttcgtctcgctcaggcgcaatcacgaatgaataacggtttggttgatgcgagtgattttgatgacgagcgtaatggctggcctgttgaacaagtctggaaagaaatgcataaacttttgccattctcaccggattcagtcgtcactcatggtgatttctcacttgataaccttatttttgacgaggggaaattaataggttgtattgatgttggacgagtcggaatcgcagaccgataccaggatcttgccatcctatggaactgcctcggtgagttttctccttcattacagaaacggctttttcaaaaatatggtattgataatcctgatatgaataaattgcagtttcatttgatgctcgatgagtttttctaactgtcagaccaagtttactcatatatactttagattgatttaaaacttcatttttaatttaaaaggatctaggtgaagatcctttttgataatctcatgaccaaaatcccttaacgtgagttttcgttccactgagcgtcagaccccgtagaaaagatcaaaggatcttcttgagatcctttttttctgcgcgtaatctgctgcttgcaaacaaaaaaaccaccgctaccagcggtggtttgtttgccggatcaagagctaccaactctttttccgaaggtaactggcttcagcagagcgcagataccaaatactgttcttctagtgtagccgtagttaggccaccacttcaagaactctgtagcaccgcctacatacctcgctctgctaatcctgttaccagtggctgctgccagtggcgataagtcgtgtcttaccgggttggactcaagacgatagttaccggataaggcgcagcggtcgggctgaacggggggttcgtgcacacagcccagcttggagcgaacgacctacaccgaactgagatacctacagcgtgagctatgagaaagcgccacgcttcccgaagggagaaaggcggacaggtatccggtaagcggcagggtcggaacaggagagcgcacgagggagcttccagggggaaacgcctggtatctttatagtcctgtcgggtttcgccacctctgacttgagcgtcgatttttgtgatgctcgtcaggggggcggagcctatggaaaaacgccagcaacgcggcctttttacggttcctggccttttgctggccttttgctcacatgt

SEQ ID NO: 13 - DNA, 6518 bp, synthetic construct
  source 1..6518: mol_type = other DNA
cctgcaggcagctgcgcgctcgctcgctcactgaggccgcccgggcaaagcccgggcgtcgggcgacctttggtcgcccggcctcagtgagcgagcgagcgcgcagagagggagtggccaactccatcactaggggttcctgcggccgcacgcgtggagctagttattaatagtaatcaattacggggtcattagttcatagcccatatatggagttccgcgttacataacttacggtaaatggcccgcctggctgaccgcccaacgacccccgcccattgacgtcaataatgacgtatgttcccatagtaacgtcaatagggactttccattgacgtcaatgggtggagtatttacggtaaactgcccacttggcagtacatcaagtgtatcatatgccaagtacgccccctattgacgtcaatgacggtaaatggcccgcctggcattatgcccagtacatgaccttatgggactttcctacttggcagtacatctacgtattagtcatcgctattaccatggtgatgcggttttggcagtacatcaatgggcgtggatagcggtttgactcacggggatttccaagtctccaccccattgacgtcaatgggagtttgttttgcaccaaaatcaacgggactttccaaaatgtcgtaacaactccgccccattgacgcaaatgggcggtaggcgtgtacggtgggaggtctatataagcagagctcgtttagtgaaccgtcagatcgcctggagacgccatccacgctgttttgacctccatagaagacaccgggaccgatccagcctccgcggattcgaatcccggccgggaacggtgcattggaacgcggattccccgtgccaagagtgacgtaagtaccgcctatagagtctataggcccacaaaaaatgctttcttcttttaatatacttttttgtttatcttatttctaatactttccctaatctctttctttcagggcaataatgatacaatgtatcatgcctctttgcaccattctaaagaataacagtgataatttctgggttaaggcaatagcaatatttctgcatataaatatttctgcatataaattgtaactgatgtaagaggtttcatattgctaatagcagctacaatccagctaccattctgcttttattttatggttgggataaggctggattattctgagtccaagctaggcccttttgctaatcatgttcatacctcttatcttcctcccacagctcctgggcaacgtgctggtctgtgtgctggcccatcactttggcaaagaattgggattcgaacatcgattgaattccccggggatcctctagagccgccaccatgggagtgaaagttctgttcgccctgatctgtatcgccgtggccgaggccgaagtgcagctggtggaatctggcggcggactggtgcaacctggcggcagcctgagactgagctgtgctgcttctggatatacatttaccaactacggcatgaattgggtcagacaggcccctggaaagggcctcgagtgggtgggctggattaacacatacaccggcgagcctacatacgccgccgacttcaagcggagattcacctttagcctggatacatctaagtccacagcctacctgcaaatgaactctcttagggccgaggacaccgccgtttactactgcgccaagtacccccactactacggtagctctcactggtacttcgacgtgtggggccagggcacactggtcaccgtgagcagcgccagcaccaagggccccagcgtgttccccctggcccccagctctaagagcaccagcggaggcaccgccgctctgggctgcctggtcaaggactactttccagagcctgtaaccgtgagctggaacagcggcgccctgaccagcggcgtgcacaccttccccgcagtgctgcagagcagcggcctgtacagcctgagcagcgtggtcacagttcctagcagcagcctgggaacacagacctacatctgcaacgtgaaccacaagcctagcaatacaaaagtggataagaaggtggaacctaagtcttgcgacaagacccacacatgccccccatgtcctgctcccgagctgctgggaggccctagtgtgttcctgttccctcctaagccaaaagataccctgatgatcagccgcacccctgaagtgacatgcgtcgtggtggacgtgtcccacgaggaccctgaagtgaagttcaactggtatgtggacggagtggaggtgcacaatgccaaaacaaagcctcgggaagagcagtacaactccacctatagagtggtgtccgtgctgaccgtgctggagcagaactggctggacggcaaggaatacaagtgcaaggttagcaacaaggccctgcctgccccaatcgagaagaccatcagcaaggccaagggccaacctagagagccccaggtgtacaccctgcctccaagcagagaggaaatgaccaaaaaccaggtgtccctgacctgtctggtgaaaggcttctaccctagcgatatcgccgtggaatgggagagcaacggccagcctgagaacaactacaagaccaccccccccgtgctggatagcgacggctccttcttcctgtactccaagctgaccgtggacaaatctcggtggcagcagggcaacgtgttcagctgcagcgtgatgcacgaggccctgcataatcactacacccagaagagcctgtctctgagccctggcaaagccaccaacttttctctgctgaagcaggctggcgacgtggaggagaacccaggacctatgggagtgaaagttctgttcgccctgatctgtatcgccgtggccgaggccgatatccagatgacccagagccctagcagcctgtccgctagcgtgggcgatagagtgaccatcacctgcagcgccagccaggacatctctaattacctgaattggtaccagcaaaagcccggcaaggcccctaaggtgctgatctacttcacaagcagcctgcacagcggcgtgccttctagattcagcggctccggcagcggcacagactttacactgacaattagcagcctgcaacctgaggacttcgccacctattactgccagcagtacagcaccgtcccatggaccttcggacagggaacaaaagtcgagatcaagcggaccgtggccgctccatctgtgttcatcttcccccccagcgacgagcagctgaagagcggaaccgcctctgtggtgtgcctgctgaacaacttctaccctagagaagccaaggtgcagtggaaggttgacaacgccctgcagtccggcaacagccaggagagcgtgacagaacaggattctaaagacagcacatactccctctctagcaccctgaccctgtccaaggccgactacgagaagcacaaggtgtacgcctgtgaagtgacccaccagggcctgagctctcctgtgaccaaaagctttaaccggggcgagtgctagtaaaagcttgcctcgagcagcgctgctcgagagatctacctgtgccttctagttgccagccatctgttgtttgcccctcccccgtgccttccttgaccctggaaggtgccactcccactgtcctttcctaataaaatgaggaaattgcatcgcattgtctgagtaggtgtcattctattctggggggtggggtggggcaggacagcaagggggaggattgggaagacaatagcaggcatgctggggatgcggtgggctctatggctgattttgtaggtaaccacgtgcggaccgagcggccgcaggaacccctagtgatggagttggccactccctctctgcgcgctcgctcgctcactgaggccgggcgaccaaaggtcgcccgacgcccgggctttgcccgggcggcctcagtgagcgagcgagcgcgcagctgcctgcaggggcgcctgatgcggtattttctccttacgcatctgtgcggtatttcacaccgcatacgtcaaagcaaccatagtacgcgccctgtagcggcgcattaagcgcggcgggtgtggtggttacgcgcagcgtgaccgctacacttgccagcgccctagcgcccgctcctttcgctttcttcccttcctttctcgccacgttcgccggctttccccgtcaagctctaaatcgggggctccctttagggttccgatttagtgctttacggcacctcgaccccaaaaaacttgatttgggtgatggttcacgtagtgggccatcgccctgatagacggtttttcgccctttgacgttggagtccacgttctttaatagtggactcttgttccaaactggaacaacactcaaccctatctcgggctattcttttgatttataagggattttgccgatttcggcctattggttaaaaaatgagctgatttaacaaaaatttaacgcgaattttaacaaaatattaacgtttacaattttatggtgcactctcagtacaatctgctctgatgccgcatagttaagccagccccgacacccgccaacacccgctgacgcgccctgacgggcttgtctgctcccggcatccgcttacagacaagctgtgaccgtctccgggagctgcatgtgtcagaggttttcaccgtcatcaccgaaacgcgcgagacgaaagggcctcgtgatacgcctatttttataggttaatgtcatgataataatggtttcttagacgtcaggtggcacttttcggggaaatgtgtgcagctctggcccgtgtctcaaaatctctgatgttacattgcacaagataaaaatatatcatcatgaacaataaaactgtctgcttacataaacagtaatacaaggggtgttatgagccatattcaacgggaaacgtcgaggccgcgattaaattccaacatggatgctgatttatatgggtataaatgggctcgcgataatgtcgggcaatcaggtgcgacaatctatcgcttgtatgggaagcccgatgcgccagagttgtttctgaaacatggcaaaggtagcgttgccaatgatgttacagatgagatggtcagactaaactggctgacggaatttatgcctcttccgaccatcaagcattttatccgtactcctgatgatgcatggttactcaccactgcgatccccggaaaaacagcattccaggtattagaagaatatcctgattcaggtgaaaatattgttgatgcgctggcagtgttcctgcgccggttgcattcgattcctgtttgtaattgtccttttaacagcgatcgcgtatttcgtctcgctcaggcgcaatcacgaatgaataacggtttggttgatgcgagtgattttgatgacgagcgtaatggctggcctgttgaacaagtctggaaagaaatgcataaacttttgccattctcaccggattcagtcgtcactcatggtgatttctcacttgataaccttatttttgacgaggggaaattaataggttgtattgatgttggacgagtcggaatcgcagaccgataccaggatcttgccatcctatggaactgcctcggtgagttttctccttcattacagaaacggctttttcaaaaatatggtattgataatcctgatatgaataaattgcagtttcatttgatgctcgatgagtttttctaactgtcagaccaagtttactcatatatactttagattgatttaaaacttcatttttaatttaaaaggatctaggtgaagatcctttttgataatctcatgaccaaaatcccttaacgtgagttttcgttccactgagcgtcagaccccgtagaaaagatcaaaggatcttcttgagatcctttttttctgcgcgtaatctgctgcttgcaaacaaaaaaaccaccgctaccagcggtggtttgtttgccggatcaagagctaccaactctttttccgaaggtaactggcttcagcagagcgcagataccaaatactgttcttctagtgtagccgtagttaggccaccacttcaagaactctgtagcaccgcctacatacctcgctctgctaatcctgttaccagtggctgctgccagtggcgataagtcgtgtcttaccgggttggactcaagacgatagttaccggataaggcgcagcggtcgggctgaacggggggttcgtgcacacagcccagcttggagcgaacgacctacaccgaactgagatacctacagcgtgagctatgagaaagcgccacgcttcccgaagggagaaaggcggacaggtatccggtaagcggcagggtcggaacaggagagcgcacgagggagcttccagggggaaacgcctggtatctttatagtcctgtcgggtttcgccacctctgacttgagcgtcgatttttgtgatgctcgtcaggggggcggagcctatggaaaaacgccagcaacgcggcctttttacggttcctggccttttgctggccttttgctcacatgt

SEQ ID NO: 14 - protein, 431 aa, synthetic construct
SDTGRPFVEMYSEIPEIIHMTEGRELVIPCRVTSPNITVTLKKFPLDTLIPDGKRIIWDSRKGFIISNATYKEIGLLTCEATVNGHLYKTNYLTHRQTNTIIDVVLSPSHGIELSVGEKLVLNCTARTELNVGIDFNWEYPSSKHQHKKLVNRDLKTQSGSEMKKFLSTLTIDGVTRSDQGLYTCAASSGLMTKKNSTFVRVHEKDKTHTCPPCPAPELLGGPSVFLFPPKPKDTLMISRTPEVTCVVVDVSHEDPEVKFNWYVDGVEVHNAKTKPREEQYNSTYRVVSVLTVLHQDWLNGKEYKCKVSNKALPAPIEKTISKAKGQPREPQVYTLPPSRDELTKNQVSLTCLVKGFYPSDIAVEWESNGQPENNYKTTPPVLDSDGSFFLYSKLTVDKSRWQQGNVFSCSVMHEALHNHYTQKSLSLSPG

SEQ ID NO: 15 - protein, 167 aa, synthetic construct
DGVEVHNAKTKPREEQYNSTYRVVSVLTVLHQDWLNGKEYKCKVSNKALPAPIEKTISKAKGQPREPQVYTLPPSRDELTKNQVSLTCLVKGFYPSDIAVEWESNGQPENNYKTTPPVLDSDGSFFLYSKLTVDKSRWQQGNVFSCSVMHEALHNHYTQKSLSLSPG

SEQ ID NO: 16 - protein, 25 aa, Human OSM
MGVLLTQRTLLSLVLALLFPSMASM

SEQ ID NO: 17 - protein, 25 aa, Human alphaherpesvirus
MGGTAARLGAVILFVVIVGLHGVRG

SEQ ID NO: 18 - protein, 21 aa, Mouse Ig Kappa
METDTLLLWVLLLWVPGSTGD

SEQ ID NO: 19 - protein, 20 aa, Human IL-2
MYRMQLLSCIALSLALVTNS

SEQ ID NO: 20 - protein, 18 aa, MAFLWLLSCWALLGTTFG
MAFLWLLSCWALLGTTFG

SEQ ID NO: 21 - protein, 15 aa, Human trypsinogen-2
MNLLLILTFVAAAVA

SEQ ID NO: 22 - protein, 16 aa, Albumin(HSA)
MKWVTFISLLFSSAYS

SEQ ID NO: 23 - protein, 26 aa, Human VEGF-A
MNFLLSWVHWSLALLLYLHHAKWSQA

SEQ ID NO: 24 - protein, 29 aa, Human Fibulin-1
MERAAPSRRVPLPLLLLGGLALLAAGVDA

SEQ ID NO: 25 - protein, 19 aa, Human Vitronectin
MAPLRPLLILALLAWVALA

SEQ ID NO: 26 - protein, 18 aa, Human Complement factor H
MRLLAKIICLMLWAICVA

SEQ ID NO: 27 - protein, 19 aa, Human Opticin
MRLLAFLSLLALVLQETGT

SEQ ID NO: 28 - protein, 26 aa, Human VEGFR-1
MVSYWDTGVLLCALLSCLLLTGSSSG

SEQ ID NO: 29 - protein, 17 aa, Gaussia luc
MGVKVLFALICIAVAEA